European Patent Specification EP 4 680 710 B1, published September 9, 2026. Title: Composition. Applicant: Unilever IP Holdings B.V. The sequence listing filed with the application follows.

SEQUENCE LISTING (1 sequence)

SEQ ID NO: 1 - protein, 368 aa, Moritella viscosa
MHKKIISPTDSLKTQHLELLESQVPHYRQAYSDRTAWLMACMSELAYVKFNPLYPNKFTEEAISSTLQKLSSTTLDPRVGKILSTLSSMSYDHVEEKKLLESELSELNGAILLDTFDCNGTQAMLVELASFNILAFRGTEATSLKDIKADIKAVTTRCETGGQVHSGFKDAFDEVCDSIVGALKAINNNKPLMITGHSLGGALATIAAKRLTFKNGIAGCYTFGSPRVGDDKWISTVKTPIYRVVNAADVVTMLPPNSIAIESASAVFSLVPYAGEVIKNTLLSKFNGYIHGGNMRYLTNCEAGNYANVKLLYSVSFLYRIKALLMGKLPVKKLAADHSISIYRQKLALVALQRKSLGDQTIKTGTKQ